European Patent Specification EP 3 107 372 B1, published November 6, 2024. Title: RESISTANCE TO GEMINIVIRUSES IN WATERMELONS. Applicant: VILMORIN & CIE. The sequence listing filed with the application follows.

SEQUENCE LISTING (26 sequences)

SEQ ID NO: 1 - DNA, 201 bp, Citrullus lanatus
ttcacaccaaatccatcctcatcttagcaaaacatcataggcaccaattttgtttgaagttaaaataccattttcatccatgtaggattcattcaaatttmgtcacaaaactctcaaacgtacaattttagtcatgttctttcctaaatttcaaaagtagtcctttttggttagtttgaggttaatatttttttatattaa

SEQ ID NO: 2 - DNA, 201 bp, Citrullus lanatus
aaactggcttcactatcatcgtccaccactaattgtggaattttcagcaccccttttttggagtcaaaactcacgtcagtaaggctctttgtgccgctttsctggaaatctatccccgcgtcacgaagctgtgttgcatgtcgaatcacttgatattctggcccggatttcttcgtttttctctccatactaccatcctta

SEQ ID NO: 3 - DNA, 201 bp, Citrullus lanatus
tgattctgtttgttttgctaactccaggacttctctttcagcttcccggaaatcgcaggtgcttagagtttggcaactttcacacgagtgctgcttctatyatcgtccattcgattctctacttcggtctcatttgcgtcttcttactcgccatcaaggttcatctctacatcggttcctaatatgacttgctccgatgcc

SEQ ID NO: 4 - DNA, 201 bp, Citrullus lanatus
tcttcttctggctatgtatctgttggtgttaatacttatcttgagcccaatgtagttttggacgactgccttgttcttaaccttccggacttctatttctyatatactgtatgaatggttatctgttaaatttgtcagtatgatatgattttgacatgacatgttttggctctttccacttctcgtttttcttggctacat

SEQ ID NO: 5 - DNA, 201 bp, Citrullus lanatus
tgatatagaatgatattacgatgcaatataagttaagagaacatataagattcgtttgttttatatttcacaattacccctttaaatgaaggcacaaactscctgaaagcacatgagtcatttagtttaacttgcgcaggtacacaatttgtgtttttccaagaaaaggggttggcctcttgtgatagggtaaatacttcg

SEQ ID NO: 6 - DNA, 201 bp, Citrullus lanatus
aataggatgtggccaagagattcccctgccttgttacacaatggacaaacggtggcatgagagactgagatggaagttctttccggttgtcagctaaattsaggttcacgattcacaccaaaatatttgttttcttagggctcttggttttccaaattgcattaaagatgctgcagaccagattggaaaaagcagcaaatg

SEQ ID NO: 7 - DNA, 201 bp, Citrullus lanatus
ccttatggcttctatgcctgatatacatcaagctgtagagtttttaagtaccacaattgtggggatagggattgaacttcccacctcaaggatagaaggtygtgccaatcaccactgagcttacctcgatttggccatcaagctgtagagttgctcacgcaagaaaaggggaaaaccagcactgccaatgtccaaaaacag

SEQ ID NO: 8 - DNA, 201 bp, Citrullus lanatus
ccagtatttctttacttattacctgcaggtgaaacttaagaatatgttgtatcacactgctcggataaattgtcttgcttggtctcctgataacaccaagrttgcaactggttcattagatacatgtgttatcatatatgaaattgacaagccagcatccagtcgtctaacaataaagggagctcatttgggtggggtgta

SEQ ID NO: 9 - DNA, 201 bp, Citrullus lanatus
ggtgaggatgggattgtttacgcaatatgtgaacttcaggaggagtgtgattcgcgtggatctttaatcttgaagaagtatatggaatataggaaattggytcagttgtcctctgaaatcaatgctcaaaacaagaatttgctagctgttggtggaccagaaggacccgaccctagggaagtcgagttatacctggaagaa

SEQ ID NO: 10 - DNA, 201 bp, Citrullus lanatus
ctacagtttcctcatttctaaactttacccaccacaaaacaaagccactactgcaagaaactgtaataattagaggggggaggtaaggaatttggtggtawgttggggaagctcaaaatagacttctggtgaatagaatagaacataaatgaagccaatttctcagacaaatcaacattgagtttccaaatcaaacacaaa

SEQ ID NO: 11 - DNA, 201 bp, Citrullus lanatus
ttcaataaatcttgaaaatagttactacaagtagtttatttattattttggaaacacactcataagtgtattttatattattttaatatgtgggatggggrcattgaacctcaagcctctagattgatagttcacgttcatgccagttgagctattactcgtatttggattttggttttggccttgtaatttttgtttgta

SEQ ID NO: 12 - DNA, 201 bp, Citrullus lanatus
ttattggctaaaggaggattatcaatttcaagtgctgttgaatggacttctaaaggatccaccattttctttttctgaggaagagaggagcatcattcatyaccgtgtgaacgggagaaaggaggcttgtctggttgtcacaaaaggcgttcccaccatttgagatgttcttttcaatgattacattctctttctcactga

SEQ ID NO: 13 - DNA, 201 bp, Citrullus lanatus
accccctgccgaacagtatgatgtccgagcggtgatgacgggggacggcagacggcggacagaaccgcgagggctgaacacgaacgcgactccggcgaacwgaggaaagcgacagacggttgcaaaaacgagagagagggagatggaatcgggcgacttgcgtgaagttgggatggagggcgtgaactgcaaccatttaaa

SEQ ID NO: 14 - DNA, 31 bp, Citrullus lanatus
gattcattcaaatttmgtcacaaaactctca

SEQ ID NO: 15 - DNA, 27 bp, Citrullus lanatus
tttgtgccgctttsctggaaatctatc

SEQ ID NO: 16 - DNA, 27 bp, Citrullus lanatus
gtgctgcttctatyatcgtccattcga

SEQ ID NO: 17 - DNA, 31 bp, Citrullus lanatus
cggacttctatttctyatatactgtatgaat

SEQ ID NO: 18 - DNA, 27 bp, Citrullus lanatus
gaaggcacaaactscctgaaagcacat

SEQ ID NO: 19 - DNA, 27 bp, Citrullus lanatus
tgtcagctaaattsaggttcacgattc

SEQ ID NO: 20 - DNA, 27 bp, Citrullus lanatus
aaggatagaaggtygtgccaatcacca

SEQ ID NO: 21 - DNA, 27 bp, Citrullus lanatus
tataggaaattggytcagttgtcctct

SEQ ID NO: 22 - DNA, 27 bp, Citrullus lanatus
gaatttggtggtawgttggggaagctc

SEQ ID NO: 23 - DNA, 23 bp, Citrullus lanatus
gtgggatggggrcattgaacctc

SEQ ID NO: 24 - DNA, 27 bp, Citrullus lanatus
gagcatcattcatyaccgtgtgaacgg

SEQ ID NO: 25 - DNA, 23 bp, Citrullus lanatus
ctccggcgaacwgaggaaagcga

SEQ ID NO: 26 - DNA, 27 bp, Citrullus lanatus
tgataacaccaagrttgcaactggttc